European Patent Application EP 4 238 993 A2, published September 6, 2023. Title: ANTIGEN-BINDING MOLECULE CAPABLE OF BINDING TO TWO OR MORE ANTIGEN MOLECULES REPEATEDLY. Applicant: CHUGAI SEIYAKU KABUSHIKI KAISHA. The sequence listing filed with the application follows.

SEQUENCE LISTING (70 sequences)

SEQ ID NO: 1 - protein, 119 aa, synthetic construct
  REGION 1..119: note = An artificially synthesized peptide sequence
QVQLQESGPGLVKPSETLSLTCAVSGYSISDDHAWSWVRQPPGEGLEWIGYISYSGITNYNPSLKGRVTISRDTSKNQFSLKLSSVTAADTAAYYCARSLARTTAMDYWGEGTLVTVSS

SEQ ID NO: 2 - protein, 107 aa, synthetic construct
  REGION 1..107: note = An artificially synthesized peptide sequence
DIQMTQSPSSLSASVGDSVTITCQASQDISSYLNWYQQKPGKAPELLIYYGSELHSGVPSRFSGSGSGTDFTFTISSLEAEDAATYYCGQGNRLPYTFGQGTKVEIE

SEQ ID NO: 3 - protein, 119 aa, synthetic construct
  REGION 1..119: note = An artificially synthesized peptide sequence
QVQLQESGPGLVKPSETLSLTCAVSGHSISHDHAHSWVRQPPGEGLEWIGYISYSGITNYNPSLKGRVTISRDTSKNQFSLKLSSVTAADTAAYYCARSLARTTAMDYWGEGTLVTVSS

SEQ ID NO: 4 - protein, 119 aa, synthetic construct
  REGION 1..119: note = An artificially synthesized peptide sequence
QVQLQESGPGLVKPSETLSLTCAVSGHSISHHHAHSWVRQPPGEGLEWIGYISYSGITHYNPHLKGRVTISRDTSKNQFSLKLSSVTAADTAAYYCARVLARITAMDHWGEGTLVTVSS

SEQ ID NO: 5 - protein, 119 aa, synthetic construct
  REGION 1..119: note = An artificially synthesized peptide sequence
QVQLQESGPGLVKPSETLSLTCAVSGYSISHDHAWSWVRQPPGEGLEWIGHISYSGITNYNPHLKGRVTISRDTSKNQFSLKLSSVTAADTAAYYCARFLARITAHDHWGEGTLVTVSS

SEQ ID NO: 6 - protein, 107 aa, synthetic construct
  REGION 1..107: note = An artificially synthesized peptide sequence
DIQMTQSPSSLSASVGDSVTITCQASQHISSHLNWYQQKPGKAPELLIYYGSHLHSGVPSRFSGSGSGTDFTFTISSLEAEDAATYYCGQGNRLPYTFGQGTKVEIE

SEQ ID NO: 7 - protein, 107 aa, synthetic construct
  REGION 1..107: note = An artificially synthesized peptide sequence
DIQMTQSPSSLSASVGDSVTITCQASQDISSHLNWYQQKPGKAPELLIYYGSHLHSGVPSRFSGSGSGTDFTFTISSLEAEDAATYYCGQGNRLPYTFGQGTKVEIE

SEQ ID NO: 8 - protein, 107 aa, synthetic construct
  REGION 1..107: note = An artificially synthesized peptide sequence
DIQMTQSPSSLSASVGDSVTITCQASQDISSHLNWYQQKPGKAPELLIYYGSHLHHGVPSRFSGSGSGTDFTFTISSLEAEDAATYYCGQGHRLPYTFGQGTKVEIE

SEQ ID NO: 9 - protein, 448 aa, synthetic construct
  REGION 1..448: note = An artificially synthesized peptide sequence
QVQLQESGPGLVRPSQTLSLTCTVSGYSITSDHAWSWVRQPPGRGLEWIGYISYSGITTYNPSLKSRVTMLRDTSKNQFSLRLSSVTAADTAVYYCARSLARTTAMDYWGQGSLVTVSSASTKGPSVFPLAPSSKSTSGGTAALGCLVKDYFPEPVTVSWNSGALTSGVHTFPAVLQSSGLYSLSSVVTVPSSSLGTQTYICNVNHKPSNTKVDKKVEPKSCDKTHTCPPCPAPELLGGPSVFLFPPKPKDTLMISRTPEVTCVVVDVSHEDPEVKFNWYVDGVEVHNAKTKPREEQYNSTYRVVSVLTVLHQDWLNGKEYKCKVSNKALPAPIEKTISKAKGQPREPQVYTLPPSRDELTKNQVSLTCLVKGFYPSDIAVEWESNGQPENNYKTTPPVLDSDGSFFLYSKLTVDKSRWQQGNVFSCSVMHEALHNHYTQKSLSLSPG

SEQ ID NO: 10 - protein, 214 aa, synthetic construct [sequence omitted]

SEQ ID NO: 11 - protein, 119 aa, synthetic construct
  REGION 1..119: note = An artificially synthesized peptide sequence
QVQLQESGPGLVKPSETLSLTCAVSGYSISDDHAWSWVRQPPGEGLEWIGYISYSGITNYNPSLKGRVTISRDTSKNQFSLKLSSVTAADTAAYYCARVLARITAMDYWGEGTLVTVSS

SEQ ID NO: 12 - protein, 107 aa, synthetic construct
  REGION 1..107: note = An artificially synthesized peptide sequence
DIQMTQSPSSLSASVGDSVTITCQASQDISSYLNWYQQKPGKAPELLIYYGSELHSGVPSRFSGSGSGTDFTFTISSLEAEDAATYYCQQGNSLPYTFGQGTKVEIE

SEQ ID NO: 13 - DNA, 1404 bp, synthetic construct
  misc_feature 1..1404: note = An artificially synthesized nucleotide sequence
  source 1..1404: mol_type = other DNA
atgggatggagctgtatcatcctcttcttggtagcaacagctacaggtgtccactcccaggtccaactgcaggagagcggtccaggtcttgtgaaacctagcgagaccctgagcctgacctgcgccgtgtctggctactcaattagcgacgatcatgcctggagctgggttcgccagccacctggagaaggtcttgagtggattggatacattagttatagtggaatcacaaactataatccatctctcaaaggcagagtgacaatatcgagagacaccagcaagaaccagttcagcctgaaactcagcagcgtgacagccgccgacaccgcggcttattattgtgcaagatccctagctcggactacggctatggactactggggtgaaggcaccctcgtcacagtctcctcagcctccaccaagggcccatcggtcttccccctggcaccctcctccaagagcacctctgggggcacagcggccctgggctgcctggtcaaggactacttccccgaaccggtgacggtgtcgtggaactcaggcgccctgaccagcggcgtgcacaccttcccggctgtcctacagtcctcaggactctactccctcagcagcgtggtgaccgtgccctccagcagcttgggcacccagacctacatctgcaacgtgaatcacaagcccagcaacaccaaggtggacaagaaagttgagcccaaatcttgtgacaaaactcacacatgcccaccgtgcccagcacctgaactcctggggggaccgtcagtcttcctcttccccccaaaacccaaggacaccctcatgatctcccggacccctgaggtcacatgcgtggtggtggacgtgagccacgaagaccctgaggtcaagttcaactggtacgtggacggcgtggaggtgcataatgccaagacaaagccgcgggaggagcagtacaacagcacgtaccgtgtggtcagcgtcctcaccgtcctgcaccaggactggctgaatggcaaggagtacaagtgcaaggtctccaacaaagccctcccagcccccatcgagaaaaccatctccaaagccaaagggcagccccgagaaccacaggtgtacaccctgcccccatcccgggatgagctgaccaagaaccaggtcagcctgacctgcctggtcaaaggcttctatcccagcgacatcgccgtggagtgggagagcaatgggcagccggagaacaactacaagaccacgcctcccgtgctggactccgacggctccttcttcctctacagcaagctcaccgtggacaagagcaggtggcagcaggggaacgtcttctcatgctccgtgatgcatgaggctctgcacaaccactacacgcagaagagcctctccctgtctccgggtaaa

SEQ ID NO: 14 - DNA, 321 bp, synthetic construct
  misc_feature 1..321: note = An artificially synthesized nucleotide sequence
  source 1..321: mol_type = other DNA
gacatccagatgacccagagcccaagcagcctgagcgccagcgtgggtgacagcgtgaccatcacctgtcaagccagccaggacatcagcagttacctgaattggtaccagcagaagccaggaaaggctccagagctgctgatctactacggctccgaactgcactctggtgtgccaagcagattcagcggtagcggtagcggtaccgacttcaccttcaccatcagcagcctcgaggcagaggacgccgctacctactactgcgggcagggtaaccggcttccatacacgttcggccaagggaccaaggtggaaatcgaa

SEQ ID NO: 15 - protein, 15 aa, synthetic construct
  REGION 1..15: note = An artificially synthesized peptide sequence
GGGGSGGGGSGGGGS

SEQ ID NO: 16 - DNA, 24 bp, synthetic construct
  misc_feature 1..24: note = An artificially syntheisized primer sequence
  source 1..24: mol_type = other DNA
ttcccaccagcctgtccgcctctg

SEQ ID NO: 17 - DNA, 24 bp, synthetic construct
  misc_feature 1..24: note = An artificially syntheisized primer sequence
  source 1..24: mol_type = other DNA
cgtgaagccaaaggccccactccc

SEQ ID NO: 18 - DNA, 32 bp, synthetic construct
  misc_feature 1..32: note = An artificially syntheisized primer sequence
  source 1..32: mol_type = other DNA
tagaattccaccatgctggccgtcggctgcgc

SEQ ID NO: 19 - DNA, 57 bp, synthetic construct
  misc_feature 1..57: note = An artificially syntheisized primer sequence
  source 1..57: mol_type = other DNA
attgcggccgcttatcagtggtgatgatgatgatgtggtaccgaagaagaatcttgc

SEQ ID NO: 20 - DNA, 1131 bp, synthetic construct
  misc_feature 1..1131: note = An artificially synthesized nucleotide sequence
  source 1..1131: mol_type = other DNA
gaattccaccatgctggccgtcggctgcgcgctgctggctgccctgctggccgcgccgggggcggcgctggccccggggggctgccctgcacaggaggtggcgagaggtgtgctgaccagtctgccaggagacagcgtgactctgacctgcccagggggagagccggaagacaatgccactgttcactgggttctcaggaagccagctgtaggctcccacctcagcagatgggctggcgtgggaaggaggctgctgctgaggtcggtgcagctccatgactctggaaactattcatgctaccgggccggccgcccggctggaactgtgcacttgctggtggatgttccccccgaggagccccagctctcctgcttccggaagagccccctcagcaacgttgtttgtgagtggggtcctcggagcaccccatctccgacgaccaaggctgtgctgttggtgaggaagtttcagaacagtccggccgaagacttccaggagccgtgccagtattcccaggagtcccagaagttctcctgccagttggcagtcccggagggagacagctctttctacatagtgtccatgtgcgtcgccagtagtgtcgggagcaagctcagcaaaactcagacctttcagggttgtggaatcttgcagcctgatccgcctgccaacatcacagtcactgccgtggccagaaacccccgctggctcagtgtcacctggcaagacccccactcctggaactcatctttctacagactacggtttgagctcagatatcgagctgaacggtcaaagacattcacaacatggatggtcaaggacctccagcatcactgtgtcatccacgacgcctggagcggcctgaggcacgtggtgcagcttcgtgcccaggaggagttcgggcaaggcgagtggagcgagtggagcccggaggccatgggcacgccttggacagaatccaggagtcctccagctgagaacgaggtgtccacccccacgcaggcacctactactaataaagatgatgataatattctctccagagattctgcaaatgcgacaagcctcccagtgcaagattcttcttcggtaccacatcatcatcatcaccactgataagcggccgc

SEQ ID NO: 21 - protein, 449 aa, synthetic construct
  REGION 1..449: note = An artificially synthesized peptide sequence
QVQLQESGPGLVKPSETLSLTCAVSGYSISHDHAWSWVRQPPGEGLEWIGHISYSGITNYNPHLQDRVTISRDTSKNQFSLKLSSVTAADTAAYYCARFLARITAHDHWGEGTLVTVSSASTKGPSVFPLAPSSKSTSGGTAALGCLVKDYFPEPVTVSWNSGALTSGVHTFPAVLQSSGLYSLSSVVTVPSSSLGTQTYICNVNHKPSNTKVDKKVEPKSCDKTHTCPPCPAPELLGGPSVFLFPPKPKDTLMISRTPEVTCVVVDVSHEDPEVKFNWYVDGVEVHNAKTKPREEQYNSTYRVVSVLTVLHQDWLNGKEYKCKVSNKALPAPIEKTISKAKGQPREPQVYTLPPSRDELTKNQVSLTCLVKGFYPSDIAVEWESNGQPENNYKTTPPVLDSDGSFFLYSKLTVDKSRWQQGNVFSCSVMHEALHNHYTQKSLSLSPGK

SEQ ID NO: 22 - protein, 449 aa, synthetic construct
  REGION 1..449: note = An artificially synthesized peptide sequence
QVQLQESGPGLVKPSETLSLTCAVSGYSISHDHAWSWVRQPPGEGLEWIGHISYSGITNYNPHLQDRVTISRDTSKNQFSLKLSSVTAADTAVYYCARFLARITAHDHWGEGTLVTVSSASTKGPSVFPLAPSSKSTSGGTAALGCLVKDYFPEPVTVSWNSGALTSGVHTFPAVLQSSGLYSLSSVVTVPSSSLGTQTYICNVNHKPSNTKVDKKVEPKSCDKTHTCPPCPAPELLGGPSVFLFPPKPKDTLMISRTPEVTCVVVDVSHEDPEVKFNWYVDGVEVHNAKTKPREEQYNSTYRVVSVLTVLHQDWLNGKEYKCKVSNKALPAPIEKTISKAKGQPREPQVYTLPPSRDELTKNQVSLTCLVKGFYPSDIAVEWESNGQPENNYKTTPPVLDSDGSFFLYSKLTVDKSRWQQGNVFSCSVMHEALHNHYTQKSLSLSPGK

SEQ ID NO: 23 - protein, 449 aa, synthetic construct
  REGION 1..449: note = An artificially synthesized peptide sequence
QVQLQESGPGLVKPSETLSLTCAVSGHSISHDHAWSWVRQPPGEGLEWIGFISYSGITNYNPSLQGRVTISRDNSKNTLYLQMNSLRAEDTAVYYCARSLARTTAMDYWGEGTLVTVSSASTKGPSVFPLAPSSKSTSGGTAALGCLVKDYFPEPVTVSWNSGALTSGVHTFPAVLQSSGLYSLSSVVTVPSSSLGTQTYICNVNHKPSNTKVDKKVEPKSCDKTHTCPPCPAPELLGGPSVFLFPPKPKDTLMISRTPEVTCVVVDVSHEDPEVKFNWYVDGVEVHNAKTKPREEQYNSTYRVVSVLTVLHQDWLNGKEYKCKVSNKALPAPIEKTISKAKGQPREPQVYTLPPSRDELTKNQVSLTCLVKGFYPSDIAVEWESNGQPENNYKTTPPVLDSDGSFFLYSKLTVDKSRWQQGNVFSCSVMHEALHNHYTQKSLSLSPGK

SEQ ID NO: 24 - protein, 449 aa, synthetic construct
  REGION 1..449: note = An artificially synthesized peptide sequence
QVQLQESGPGLVKPSETLSLTCAVSGHSISHDHAWSWVRQPPGEGLEWIGFISYSGITNYNPTLQGRVTISRDNSKNTLYLQMNSLRAEDTAVYYCARSLARTTAMDYWGEGTLVTVSSASTKGPSVFPLAPSSKSTSGGTAALGCLVKDYFPEPVTVSWNSGALTSGVHTFPAVLQSSGLYSLSSVVTVPSSSLGTQTYICNVNHKPSNTKVDKKVEPKSCDKTHTCPPCPAPELLGGPSVFLFPPKPKDTLMISRTPEVTCVVVDVSHEDPEVKFNWYVDGVEVHNAKTKPREEQYNSTYRVVSVLTVLHQDWLNGKEYKCKVSNKALPAPIEKTISKAKGQPREPQVYTLPPSRDELTKNQVSLTCLVKGFYPSDIAVEWESNGQPENNYKTTPPVLDSDGSFFLYSKLTVDKSRWQQGNVFSCSVMHEALHNHYTQKSLSLSPGK

SEQ ID NO: 25 - protein, 214 aa, synthetic construct
  REGION 1..214: note = An artificially synthesized peptide sequence
DIQMTQSPSSLSASVGDSVTITCQASRDISSHLNWYQQKPGKAPELLIYYGSHLLSGVPSRFSGSGSGTDFTFTISSLEAEDAATYYCGQGNRLPYTFGQGTKVEIERTVAAPSVFIFPPSDEQLKSGTASVVCLLNNFYPREAKVQWKVDNALQSGNSQESVTEQDSKDSTYSLSSTLTLSKADYEKHKVYACEVTHQGLSSPVTKSFNRGEC

SEQ ID NO: 26 - protein, 214 aa, synthetic construct
  REGION 1..214: note = An artificially synthesized peptide sequence
DIQMTQSPSSLSASVGDSVTITCQASRDISSHLNWYQQKPGKAPELLIYYGSHLESGVPSRFSGSGSGTDFTFTISSLEAEDAATYYCGQGNRLPYTFGQGTKVEIERTVAAPSVFIFPPSDEQLKSGTASVVCLLNNFYPREAKVQWKVDNALQSGNSQESVTEQDSKDSTYSLSSTLTLSKADYEKHKVYACEVTHQGLSSPVTKSFNRGEC

SEQ ID NO: 27 - protein, 214 aa, synthetic construct
  REGION 1..214: note = An artificially synthesized peptide sequence
DIQMTQSPSSLSASVGDSVTITCQASTDISSHLNWYQQKPGKAPELLIYYGSHLLSGVPSRFSGSGSGTDFTFTISSLEAEDAATYYCGQGNRLPYTFGQGTKVEIERTVAAPSVFIFPPSDEQLKSGTASVVCLLNNFYPREAKVQWKVDNALQSGNSQESVTEQDSKDSTYSLSSTLTLSKADYEKHKVYACEVTHQGLSSPVTKSFNRGEC

SEQ ID NO: 28 - protein, 326 aa, Homo sapiens
ASTKGPSVFPLAPCSRSTSESTAALGCLVKDYFPEPVTVSWNSGALTSGVHTFPAVLQSSGLYSLSSVVTVPSSNFGTQTYTCNVDHKPSNTKVDKTVERKCCVECPPCPAPPVAGPSVFLFPPKPKDTLMISRTPEVTCVVVDVSHEDPEVQFNWYVDGVEVHNAKTKPREEQFNSTFRVVSVLTVVHQDWLNGKEYKCKVSNKGLPAPIEKTISKTKGQPREPQVYTLPPSREEMTKNQVSLTCLVKGFYPSDIAVEWESNGQPENNYKTTPPMLDSDGSFFLYSKLTVDKSRWQQGNVFSCSVMHEALHNHYTQKSLSLSPGK

SEQ ID NO: 29 - protein, 324 aa, synthetic construct
  REGION 1..324: note = An artificially synthesized peptide sequence
ASTKGPSVFPLAPCSRSTSESTAALGCLVKDYFPEPVTVSWNSGALTSGVHTFPAVLQSSGLYSLSSVVTVPSSNFGTQTYTCNVDHKPSNTKVDKTVERKCCVECPPCPAPPVAGPSVFLFPPKPKDTLMISRTPEVTCVVVDVSHEDPEVQFNWYVDGVEVHNAKTKPREEQFNSTFRVVSVLTVVHQDWLNGKEYKCKVSNKGLPAPIEKTISKTKGQPREPQVYTLPPSREEMTKNQVSLTCLVKGFYPSDIAVEWESNGQPENNYKTTPPMLDSDGSFFLYSKLTVDKSRWQQGNVFSCSVMHEALHNHYTQKSLSLSP

SEQ ID NO: 30 - protein, 324 aa, synthetic construct
  REGION 1..324: note = An artificially synthesized peptide sequence
ASTKGPSVFPLAPSSKSTSGGTAALGCLVKDYFPEPVTVSWNSGALTSGVHTFPAVLQSSGLYSLSSVVTVPSSNFGTQTYTCNVDHKPSNTKVDKTVERKSCVECPPCPAPPVAGPSVFLFPPKPKDTLMISRTPEVTCVVVDVSQEDPEVQFNWYVDGVEVHNAKTKPREEQFNSTFRVVSVLTVVHQDWLNGKEYKCKVSNKGLPAPIEKTISKTKGQPREPQVYTLPPSQEEMTKNQVSLTCLVKGFYPSDIAVEWESNGQPENNYKTTPPMLDSDGSFFLYSKLTVDKSRWQEGNVFSCSVMHEALHNHYTQKSLSLSP

SEQ ID NO: 31 - protein, 326 aa, synthetic construct
  REGION 1..326: note = An artificially synthesized peptide sequence
ASTKGPSVFPLAPCSRSTSESTAALGCLVKDYFPEPVTVSWNSGALTSGVHTFPAVLQSSGLYSLSSVVTVPSSNFGTQTYTCNVDHKPSNTKVDKTVERKCCVECPPCPAPPVAGPSVFLFPPKPKDTLMISRTPEVTCVVVDVSHEDPEVQFNWYVDGVEVHNAKTKPREEQFNSTFRVVSVLTVVHQDWLNGKEYKCKVSNKGLPAPIEKTISKTKGQPREPQVYTLPPSREEMTKNQVSLTCLVKGFYPSDIAVEWESNGQPENNYKTTPPMLDSDGSFFLYSKLTVDKSRWQQGNVFSCSVMHEALHAHYTQKSLSLSPGK

SEQ ID NO: 32 - protein, 324 aa, synthetic construct
  REGION 1..324: note = An artificially synthesized peptide sequence
ASTKGPSVFPLAPSSKSTSGGTAALGCLVKDYFPEPVTVSWNSGALTSGVHTFPAVLQSSGLYSLSSVVTVPSSNFGTQTYTCNVDHKPSNTKVDKTVERKSCVECPPCPAPPVAGPSVFLFPPKPKDTLMISRTPEVTCVVVDVSQEDPEVQFNWYVDGVEVHNAKTKPREEQFNSTFRVVSVLTVVHQDWLNGKEYKCKVSNKGLPAPIEKTISKTKGQPREPQVYTLPPSQEEMTKNQVSLTCLVKGFYPSDIAVEWESNGQPENNYKTTPPMLDSDGSFFLYSKLTVDKSRWQEGNVFSCSVMHEALHAHYTQKSLSLSP

SEQ ID NO: 33 - protein, 443 aa, synthetic construct
  REGION 1..443: note = An artificially synthesized peptide sequence
QVQLQESGPGLVKPSETLSLTCAVSGHSISHDHAWSWVRQPPGEGLEWIGFISYSGITNYNPSLQGRVTISRDNSKNTLYLQMNSLRAEDTAVYYCARSLARTTAMDYWGEGTLVTVSSASTKGPSVFPLAPCSRSTSESTAALGCLVKDYFPEPVTVSWNSGALTSGVHTFPAVLQSSGLYSLSSVVTVPSSNFGTQTYTCNVDHKPSNTKVDKTVERKCCVECPPCPAPPVAGPSVFLFPPKPKDTLMISRTPEVTCVVVDVSHEDPEVQFNWYVDGVEVHNAKTKPREEQFNSTFRVVSVLTVVHQDWLNGKEYKCKVSNKGLPAPIEKTISKTKGQPREPQVYTLPPSREEMTKNQVSLTCLVKGFYPSDIAVEWESNGQPENNYKTTPPMLDSDGSFFLYSKLTVDKSRWQQGNVFSCSVMHEALHNHYTQKSLSLSP

SEQ ID NO: 34 - protein, 443 aa, synthetic construct
  REGION 1..443: note = An artificially synthesized peptide sequence
QVQLQESGPGLVKPSETLSLTCAVSGHSISHDHAWSWVRQPPGEGLEWIGFISYSGITNYNPSLQGRVTISRDNSKNTLYLQMNSLRAEDTAVYYCARSLARTTAMDYWGEGTLVTVSSASTKGPSVFPLAPSSKSTSGGTAALGCLVKDYFPEPVTVSWNSGALTSGVHTFPAVLQSSGLYSLSSVVTVPSSNFGTQTYTCNVDHKPSNTKVDKTVERKSCVECPPCPAPPVAGPSVFLFPPKPKDTLMISRTPEVTCVVVDVSQEDPEVQFNWYVDGVEVHNAKTKPREEQFNSTFRVVSVLTVVHQDWLNGKEYKCKVSNKGLPAPIEKTISKTKGQPREPQVYTLPPSQEEMTKNQVSLTCLVKGFYPSDIAVEWESNGQPENNYKTTPPMLDSDGSFFLYSKLTVDKSRWQEGNVFSCSVMHEALHNHYTQKSLSLSP

SEQ ID NO: 35 - protein, 443 aa, synthetic construct
  REGION 1..443: note = An artificially synthesized peptide sequence
QVQLQESGPGLVKPSETLSLTCAVSGHSISHDHAWSWVRQPPGEGLEWIGFISYSGITNYNPSLQGRVTISRDNSKNTLYLQMNSLRAEDTAVYYCARSLARTTAMDYWGEGTLVTVSSASTKGPSVFPLAPSSKSTSGGTAALGCLVKDYFPEPVTVSWNSGALTSGVHTFPAVLQSSGLYSLSSVVTVPSSNFGTQTYTCNVDHKPSNTKVDKTVERKSCVECPPCPAPPVAGPSVFLFPPKPKDTLMISRTPEVTCVVVDVSQEDPEVQFNWYVDGVEVHNAKTKPREEQFNSTFRVVSVLTVVHQDWLNGKEYKCKVSNKGLPAPIEKTISKTKGQPREPQVYTLPPSQEEMTKNQVSLTCLVKGFYPSDIAVEWESNGQPENNYKTTPPMLDSDGSFFLYSKLTVDKSRWQEGNVFSCSVMHEALHAHYTQKSLSLSP

SEQ ID NO: 36 - protein, 445 aa, synthetic construct
  REGION 1..445: note = An artificially synthesized peptide sequence
QVQLQESGPGLVKPSETLSLTCAVSGYSISHDHAWSWVRQPPGEGLEWIGHISYSGITNYNPHLQDRVTISRDTSKNQFSLKLSSVTAADTAVYYCARFLARITAHDHWGEGTLVTVSSASTKGPSVFPLAPCSRSTSESTAALGCLVKDYFPEPVTVSWNSGALTSGVHTFPAVLQSSGLYSLSSVVTVPSSNFGTQTYTCNVDHKPSNTKVDKTVERKCCVECPPCPAPPVAGPSVFLFPPKPKDTLMISRTPEVTCVVVDVSHEDPEVQFNWYVDGVEVHNAKTKPREEQFNSTFRVVSVLTVVHQDWLNGKEYKCKVSNKGLPAPIEKTISKTKGQPREPQVYTLPPSREEMTKNQVSLTCLVKGFYPSDIAVEWESNGQPENNYKTTPPMLDSDGSFFLYSKLTVDKSRWQQGNVFSCSVMHEALHAHYTQKSLSLSPGK

SEQ ID NO: 37 - protein, 443 aa, synthetic construct
  REGION 1..443: note = An artificially synthesized peptide sequence
QVQLQESGPGLVKPSETLSLTCAVSGYSISHDHAWSWVRQPPGEGLEWIGHISYSGITNYNPHLQDRVTISRDTSKNQFSLKLSSVTAADTAVYYCARFLARITAHDHWGEGTLVTVSSASTKGPSVFPLAPSSKSTSGGTAALGCLVKDYFPEPVTVSWNSGALTSGVHTFPAVLQSSGLYSLSSVVTVPSSNFGTQTYTCNVDHKPSNTKVDKTVERKSCVECPPCPAPPVAGPSVFLFPPKPKDTLMISRTPEVTCVVVDVSQEDPEVQFNWYVDGVEVHNAKTKPREEQFNSTFRVVSVLTVVHQDWLNGKEYKCKVSNKGLPAPIEKTISKTKGQPREPQVYTLPPSQEEMTKNQVSLTCLVKGFYPSDIAVEWESNGQPENNYKTTPPMLDSDGSFFLYSKLTVDKSRWQEGNVFSCSVMHEALHAHYTQKSLSLSP

SEQ ID NO: 38 - protein, 445 aa, synthetic construct
  REGION 1..445: note = An artificially synthesized peptide sequence
QVQLQESGPGLVKPSETLSLTCAVSGHSISHDHAWSWVRQPPGEGLEWIGFISYSGITNYNPTLQGRVTISRDNSKNTLYLQMNSLRAEDTAVYYCARSLARTTAMDYWGEGTLVTVSSASTKGPSVFPLAPCSRSTSESTAALGCLVKDYFPEPVTVSWNSGALTSGVHTFPAVLQSSGLYSLSSVVTVPSSNFGTQTYTCNVDHKPSNTKVDKTVERKCCVECPPCPAPPVAGPSVFLFPPKPKDTLMISRTPEVTCVVVDVSHEDPEVQFNWYVDGVEVHNAKTKPREEQFNSTFRVVSVLTVVHQDWLNGKEYKCKVSNKGLPAPIEKTISKTKGQPREPQVYTLPPSREEMTKNQVSLTCLVKGFYPSDIAVEWESNGQPENNYKTTPPMLDSDGSFFLYSKLTVDKSRWQQGNVFSCSVMHEALHAHYTQKSLSLSPGK

SEQ ID NO: 39 - protein, 443 aa, synthetic construct
  REGION 1..443: note = An artificially synthesized peptide sequence
QVQLQESGPGLVKPSETLSLTCAVSGHSISHDHAWSWVRQPPGEGLEWIGFISYSGITNYNPTLQGRVTISRDNSKNTLYLQMNSLRAEDTAVYYCARSLARTTAMDYWGEGTLVTVSSASTKGPSVFPLAPSSKSTSGGTAALGCLVKDYFPEPVTVSWNSGALTSGVHTFPAVLQSSGLYSLSSVVTVPSSNFGTQTYTCNVDHKPSNTKVDKTVERKSCVECPPCPAPPVAGPSVFLFPPKPKDTLMISRTPEVTCVVVDVSQEDPEVQFNWYVDGVEVHNAKTKPREEQFNSTFRVVSVLTVVHQDWLNGKEYKCKVSNKGLPAPIEKTISKTKGQPREPQVYTLPPSQEEMTKNQVSLTCLVKGFYPSDIAVEWESNGQPENNYKTTPPMLDSDGSFFLYSKLTVDKSRWQEGNVFSCSVMHEALHAHYTQKSLSLSP

SEQ ID NO: 40 - protein, 6 aa, synthetic construct
  REGION 1..6: note = An artificially synthesized peptide sequence
HDHAWS

SEQ ID NO: 41 - protein, 16 aa, synthetic construct
  REGION 1..16: note = An artificially synthesized peptide sequence
HISYSGITNYNPHLQD

SEQ ID NO: 42 - protein, 16 aa, synthetic construct
  REGION 1..16: note = An artificially synthesized peptide sequence
FISYSGITNYNPSLQG

SEQ ID NO: 43 - protein, 16 aa, synthetic construct
  REGION 1..16: note = An artificially synthesized peptide sequence
FISYSGITNYNPTLQG

SEQ ID NO: 44 - protein, 10 aa, synthetic construct
  REGION 1..10: note = An artificially synthesized peptide sequence
FLARITAHDH

SEQ ID NO: 45 - protein, 10 aa, synthetic construct
  REGION 1..10: note = An artificially synthesized peptide sequence
SLARTTAMDY

SEQ ID NO: 46 - protein, 30 aa, synthetic construct
  REGION 1..30: note = An artificially synthesized peptide sequence
QVQLQESGPGLVKPSETLSLTCAVSGYSIS

SEQ ID NO: 47 - protein, 30 aa, synthetic construct
  REGION 1..30: note = An artificially synthesized peptide sequence
QVQLQESGPGLVKPSETLSLTCAVSGHSIS

SEQ ID NO: 48 - protein, 14 aa, synthetic construct
  REGION 1..14: note = An artificially synthesized peptide sequence
WVRQPPGEGLEWIG

SEQ ID NO: 49 - protein, 32 aa, synthetic construct
  REGION 1..32: note = An artificially synthesized peptide sequence
RVTISRDTSKNQFSLKLSSVTAADTAAYYCAR

SEQ ID NO: 50 - protein, 32 aa, synthetic construct
  REGION 1..32: note = An artificially synthesized peptide sequence
RVTISRDTSKNQFSLKLSSVTAADTAVYYCAR

SEQ ID NO: 51 - protein, 32 aa, synthetic construct
  REGION 1..32: note = An artificially synthesized peptide sequence
RVTISRDNSKNTLYLQMNSLRAEDTAVYYCAR

SEQ ID NO: 52 - protein, 11 aa, synthetic construct
  REGION 1..11: note = An artificially synthesized peptide sequence
WGEGTLVTVSS

SEQ ID NO: 53 - protein, 11 aa, synthetic construct
  REGION 1..11: note = An artificially synthesized peptide sequence
QASRDISSHLN

SEQ ID NO: 54 - protein, 11 aa, synthetic construct
  REGION 1..11: note = An artificially synthesized peptide sequence
QASTDISSHLN

SEQ ID NO: 55 - protein, 7 aa, synthetic construct
  REGION 1..7: note = An artificially synthesized peptide sequence
YGSHLLS

SEQ ID NO: 56 - protein, 7 aa, synthetic construct
  REGION 1..7: note = An artificially synthesized peptide sequence
YGSHLES

SEQ ID NO: 57 - protein, 9 aa, synthetic construct
  REGION 1..9: note = An artificially synthesized peptide sequence
GQGNRLPYT

SEQ ID NO: 58 - protein, 23 aa, synthetic construct
  REGION 1..23: note = An artificially synthesized peptide sequence
DIQMTQSPSSLSASVGDSVTITC

SEQ ID NO: 59 - protein, 15 aa, synthetic construct
  REGION 1..15: note = An artificially synthesized peptide sequence
WYQQKPGKAPELLIY

SEQ ID NO: 60 - protein, 32 aa, synthetic construct
  REGION 1..32: note = An artificially synthesized peptide sequence
GVPSRFSGSGSGTDFTFTISSLEAEDAATYYC

SEQ ID NO: 61 - protein, 10 aa, synthetic construct
  REGION 1..10: note = An artificially synthesized peptide sequence
FGQGTKVEIE

SEQ ID NO: 62 - protein, 449 aa, synthetic construct
  REGION 1..449: note = An artificially synthesized peptide sequence
EVQLVESGGKLLKPGGSLKLSCAASGFTFSSFAMSWFRQSPEKRLEWVAEISSGGSYTYYPDTVTGRFTISRDNAKNTLYLEMSSLRSEDTAMYYCARGLWGYYALDYWGQGTSVTVSSASTKGPSVFPLAPSSKSTSGGTAALGCLVKDYFPEPVTVSWNSGALTSGVHTFPAVLQSSGLYSLSSVVTVPSSSLGTQTYICNVNHKPSNTKVDKKVEPKSCDKTHTCPPCPAPELLGGPSVFLFPPKPKDTLMISRTPEVTCVVVDVSHEDPEVKFNWYVDGVEVHNAKTKPREEQYNSTYRVVSVLTVLHQDWLNGKEYKCKVSNKALPAPIEKTISKAKGQPREPQVYTLPPSRDELTKNQVSLTCLVKGFYPSDIAVEWESNGQPENNYKTTPPVLDSDGSFFLYSKLTVDKSRWQQGNVFSCSVMHEALHNHYTQKSLSLSPGK

SEQ ID NO: 63 - protein, 213 aa, synthetic construct
  REGION 1..213: note = An artificially synthesized peptide sequence
QIVLIQSPAIMSASPGEKVTMTCSASSSVSYMYWYQQKPGSSPRLLIYDTSNLASGVPVRFSGSGSGTSYSLTISRMEAEDAATYYCQQWSGYPYTFGGGTKLEIKRTVAAPSVFIFPPSDEQLKSGTASVVCLLNNFYPREAKVQWKVDNALQSGNSQESVTEQDSKDSTYSLSSTLTLSKADYEKHKVYACEVTHQGLSSPVTKSFNRGEC

SEQ ID NO: 64 - protein, 449 aa, synthetic construct
  REGION 1..449: note = An artificially synthesized peptide sequence
EVQLVESGGKLLKPGGSLKLSCAASGFTFSSHAMSWFRQSPEKRLEWVAEISSGGSYTYHPHTVTGRFTISRDNAKNTLYLEMSSLRSEDTAMYYCARGLWGHYALDYWGQGTSVTVSSASTKGPSVFPLAPSSKSTSGGTAALGCLVKDYFPEPVTVSWNSGALTSGVHTFPAVLQSSGLYSLSSVVTVPSSSLGTQTYICNVNHKPSNTKVDKKVEPKSCDKTHTCPPCPAPELLGGPSVFLFPPKPKDTLMISRTPEVTCVVVDVSHEDPEVKFNWYVDGVEVHNAKTKPREEQYNSTYRVVSVLTVLHQDWLNGKEYKCKVSNKALPAPIEKTISKAKGQPREPQVYTLPPSRDELTKNQVSLTCLVKGFYPSDIAVEWESNGQPENNYKTTPPVLDSDGSFFLYSKLTVDKSRWQQGNVFSCSVMHEALHNHYTQKSLSLSPGK

SEQ ID NO: 65 - protein, 213 aa, synthetic construct
  REGION 1..213: note = An artificially synthesized peptide sequence
QIVLIQSPAIMSASPGEKVTMTCSASSSVSYMYWYQQKPGSSPRLLIYDTSNHASGVPVRFSGSGSGTSYSLTISRMEAEDAATYYCQHWSGHPYTFGGGTKLEIKRTVAAPSVFIFPPSDEQLKSGTASVVCLLNNFYPREAKVQWKVDNALQSGNSQESVTEQDSKDSTYSLSSTLTLSKADYEKHKVYACEVTHQGLSSPVTKSFNRGEC

SEQ ID NO: 66 - protein, 213 aa, synthetic construct
  REGION 1..213: note = An artificially synthesized peptide sequence
QIVLIQSPAIMSASPGEKVTMTCSASSSVSYMYWYQQKPGSSPRLLIYDTSHHASGVPVRFSGSGSGTSYSLTISRMEAEDAATYYCQHWSGHPYTFGGGTKLEIKRTVAAPSVFIFPPSDEQLKSGTASVVCLLNNFYPREAKVQWKVDNALQSGNSQESVTEQDSKDSTYSLSSTLTLSKADYEKHKVYACEVTHQGLSSPVTKSFNRGEC

SEQ ID NO: 67 - protein, 456 aa, synthetic construct
  REGION 1..456: note = An artificially synthesized peptide sequence
QVQLVQSGAEVKKPGASVKVSCKASGYTFTGYYMHWVRQAPGQGLEWMGWINPNSGGTNYAQKFQGRVTMTRDTSISTAYMELSRLRSDDTAVYYCAREDVVPAAMSFYYGMDVWGRGTLVTVSSASTKGPSVFPLAPSSKSTSGGTAALGCLVKDYFPEPVTVSWNSGALTSGVHTFPAVLQSSGLYSLSSVVTVPSSSLGTQTYICNVNHKPSNTKVDKKVEPKSCDKTHTCPPCPAPELLGGPSVFLFPPKPKDTLMISRTPEVTCVVVDVSHEDPEVKFNWYVDGVEVHNAKTKPREEQYNSTYRVVSVLTVLHQDWLNGKEYKCKVSNKALPAPIEKTISKAKGQPREPQVYTLPPSRDELTKNQVSLTCLVKGFYPSDIAVEWESNGQPENNYKTTPPVLDSDGSFFLYSKLTVDKSRWQQGNVFSCSVMHEALHNHYTQKSLSLSPGKG

SEQ ID NO: 68 - protein, 214 aa, synthetic construct
  REGION 1..214: note = An artificially synthesized peptide sequence
LPVLTQPPSVSVAPGQTARITCGGNNIGSKTVYWYQQEPGQAPVLVVYDDTDRPAGIPERFSGANSGNTATLTISRVEAGDEADYYCQVWDSSTDHGVFGGGTKLTVLGQPKANPTVTLFPPSSEELQANKATLVCLISDFYPGAVTVAWKADGSPVKAGVETTKPSKQSNNKYAASSYLSLTPEQWKSHRSYSCQVTHEGSTVEKTVAPTECS

SEQ ID NO: 69 - protein, 456 aa, synthetic construct
  REGION 1..456: note = An artificially synthesized peptide sequence
QVQLVQSGAEVKKPGASVKVSCKASGYTFTGYHMHWVRQAPGQGLEWMGWINPNSGGTNYAQKFQGRVTMTRDTSISTAYMELSRLRSDDTAVYYCAREDVVPAAMSFYYGMDVWGRGTLVTVSSASTKGPSVFPLAPSSKSTSGGTAALGCLVKDYFPEPVTVSWNSGALTSGVHTFPAVLQSSGLYSLSSVVTVPSSSLGTQTYICNVNHKPSNTKVDKKVEPKSCDKTHTCPPCPAPELLGGPSVFLFPPKPKDTLMISRTPEVTCVVVDVSHEDPEVKFNWYVDGVEVHNAKTKPREEQYNSTYRVVSVLTVLHQDWLNGKEYKCKVSNKALPAPIEKTISKAKGQPREPQVYTLPPSRDELTKNQVSLTCLVKGFYPSDIAVEWESNGQPENNYKTTPPVLDSDGSFFLYSKLTVDKSRWQQGNVFSCSVMHEALHNHYTQKSLSLSPGKG

SEQ ID NO: 70 - protein, 449 aa, synthetic construct
  REGION 1..449: note = An artificially synthesized peptide sequence
QVQLQESGPGLVKPSETLSLTCAVSGYSISDDQAWSWVRQPPGEGLEWIGYISYSGITNYNPSLKGRVTISRDTSKNQFSLKLSSVTAADTAAYYCARSLARTTAMDYWGEGTLVTVSSASTKGPSVFPLAPSSKSTSGGTAALGCLVKDYFPEPVTVSWNSGALTSGVHTFPAVLQSSGLYSLSSVVTVPSSSLGTQTYICNVNHKPSNTKVDKKVEPKSCDKTHTCPPCPAPELLGGPSVFLFPPKPKDTLMISRTPEVTCVVVDVSHEDPEVKFNWYVDGVEVHNAKTKPREEQYNSTYRVVSVLTVLHQDWLNGKEYKCKVSNKALPAPIEKTISKAKGQPREPQVYTLPPSRDELTKNQVSLTCLVKGFYPSDIAVEWESNGQPENNYKTTPPVLDSDGSFFLYSKLTVDKSRWQQGNVFSCSVMHEALHNHYTQKSLSLSPGK